European Patent Specification EP 3 284 832 B1, published June 7, 2023. Title: Method for Generating Aptamers with Improved Off-Rates. Applicant: Somalogic, Inc. Application EP 08782010.6. The sequence listing filed with the application follows.

SEQUENCE LISTING (23 sequences)

SEQ ID NO: 1 - DNA, 79 bp, Artificial
  source: /note= "Description of artificial sequence: Synthetic"
  misc_feature 2, 4: t is dT-biotin
  misc_feature (23)..(62): n is a, c, g, or t
atatgtcttcttgtcgtttcgcnnnnnnnnnnnnnnnnnnnnnnnnnnnnnnnnnnnnnnnnggtggagtgtggtgagg

SEQ ID NO: 2 - DNA, 25 bp, Artificial
  source: /note= "Description of artificial sequence: Synthetic"
atatatatcctcaccacactccacc

SEQ ID NO: 3 - DNA, 30 bp, Artificial
  source: /note= "Description of artificial sequence: Synthetic"
  misc_feature 2, 4: t is dT-biotin
atatttttttttgtcttcttgtcgtttcgc

SEQ ID NO: 4 - DNA, 78 bp, Artificial
  source: /note= "Description of artificial sequence: Synthetic"
  misc_feature 2, 4: t is dT-biotin
  misc_feature (22)..(61): n is a, c, g, or t
atatccgtcctcctctccgtcnnnnnnnnnnnnnnnnnnnnnnnnnnnnnnnnnnnnnnnngggacactgggtgcagg

SEQ ID NO: 5 - DNA, 25 bp, Artificial
  source: /note= "Description of artificial sequence: Synthetic"
atatatatcctgcacccagtgtccc

SEQ ID NO: 6 - DNA, 29 bp, Artificial
  source: /note= "Description of artificial sequence: Synthetic"
  misc_feature 2, 4: t is dT-biotin
atatttttttttccgtcctcctctccgtc

SEQ ID NO: 7 - DNA, 18 bp, Artificial
  source: /note= "Description of artificial sequence: Synthetic"
gtcttcttgtcgtttcgc

SEQ ID NO: 8 - DNA, 76 bp, Artificial
  source: /note= "Description of artificial sequence: Synthetic"
  misc_feature 2, 4: t is dT-biotin
  misc_feature (20)..(59): n is a, c, g, or t
atatcccgctcgtcgtctgnnnnnnnnnnnnnnnnnnnnnnnnnnnnnnnnnnnnnnnncaggcagacggtcactc

SEQ ID NO: 9 - DNA, 25 bp, Artificial
  source: /note= "Description of artificial sequence: Synthetic"
atatatatgagtgaccgtctgcctg

SEQ ID NO: 10 - DNA, 25 bp, Artificial
  source: /note= "Description of artificial sequence: Synthetic"
atatatatgagtgaccgtctgcctg

SEQ ID NO: 11 - DNA, 25 bp, Artificial
  source: /note= "Description of artificial sequence: Synthetic"
atatatatgagtgaccgtctgcctg

SEQ ID NO: 12 - DNA, 25 bp, Artificial
  source: /note= "Description of artificial sequence: Synthetic"
atatatatgagtgaccgtctgcctg

SEQ ID NO: 13 - DNA, 25 bp, Artificial
  source: /note= "Description of artificial sequence: Synthetic"
atatatatgagtgaccgtctgcctg

SEQ ID NO: 14 - DNA, 23 bp, Artificial
  source: /note= "Description of artificial sequence: Synthetic"
ttttttttcccgctcgtcgtctg

SEQ ID NO: 15 - DNA, 27 bp, Artificial
  source: /note= "Description of artificial sequence: Synthetic"
  misc_feature 2, 4: t is dT-biotin
atatttttttttcccgctcgtcgtctg

SEQ ID NO: 16 - DNA, 79 bp, Artificial
  source: /note= "Description of artificial sequence: Synthetic"
  misc_feature 2, 4: t is dT-biotin
  misc_feature (23)..(62): n is a, c, g, or t
atatgtgtctgtctgtgtcctcnnnnnnnnnnnnnnnnnnnnnnnnnnnnnnnnnnnnnnnnggtggagtgtggtgagg

SEQ ID NO: 17 - DNA, 25 bp, Artificial
  source: /note= "Description of artificial sequence: Synthetic"
atatatatcctcaccacactccacc

SEQ ID NO: 18 - DNA, 25 bp, Artificial
  source: /note= "Description of artificial sequence: Synthetic"
atatatatcctcaccacactccacc

SEQ ID NO: 19 - DNA, 25 bp, Artificial
  source: /note= "Description of artificial sequence: Synthetic"
atatatatcctcaccacactccacc

SEQ ID NO: 20 - DNA, 25 bp, Artificial
  source: /note= "Description of artificial sequence: Synthetic"
atatatatcctcaccacactccacc

SEQ ID NO: 21 - DNA, 25 bp, Artificial
  source: /note= "Description of artificial sequence: Synthetic"
atatatatcctcaccacactccacc

SEQ ID NO: 22 - DNA, 26 bp, Artificial
  source: /note= "Description of artificial sequence: Synthetic"
ttttttttgtgtctgtctgtgtcctc

SEQ ID NO: 23 - DNA, 30 bp, Artificial
  source: /note= "Description of artificial sequence: Synthetic"
  misc_feature 2, 4: t is dT-biotin
atatttttttttgtgtctgtctgtgtcctc